European Patent Specification EP 3 572 087 B9, published October 4, 2023. Title: Composition for Preventing or Treating Osteoarthritis Comprising Sialyllactose or Salts Thereof. Applicant: AJOU UNIVERSITY INDUSTRY-ACADEMIC COOPERATION FOUNDATION. The sequence listing filed with the application follows.

SEQUENCE LISTING (8 sequences)

SEQ ID NO: 1 - DNA, 22 bp, Artificial Sequence
  Col2a1-S
cacactggtaagtggggcaaga

SEQ ID NO: 2 - DNA, 23 bp, Artificial Sequence
  Col2a1-AS
ggattgtgttgtttcagggttcg

SEQ ID NO: 3 - DNA, 19 bp, Artificial Sequence
  Gapdh-S
tcactgccacccagaagac

SEQ ID NO: 4 - DNA, 19 bp, Artificial Sequence
  Gapdh-AS
tgtaggccatgaggtccac

SEQ ID NO: 5 - DNA, 21 bp, Artificial Sequence
  Mmp3-S
tcctgatgttggtggcttcag

SEQ ID NO: 6 - DNA, 21 bp, Artificial Sequence
  Mmp3-AS
tgtcttggcaaatccggtgta

SEQ ID NO: 7 - DNA, 23 bp, Artificial Sequence
  Mmp13-S
tgatggaccttctggtcttctgg

SEQ ID NO: 8 - DNA, 23 bp, Artificial Sequence
  Mmp13-AS
catccacatggttgggaagttct